European Patent Application EP 4 722 235 A1, published April 8, 2026. Title: 多肽及其偶联物和应用. Applicant: 南通壹宸生物医药科技有限公司. The sequence listing filed with the application follows.

SEQUENCE LISTING (1 sequence)

SEQ ID NO: 1 - protein, 99 aa, synthetic construct
  source 1..99: note; note (original language) = 多肽
  VARIANT 14: note; note (original language) = 能够与修饰物进行偶联，且在肿瘤微环境中能够与修饰物解偶联，释放多肽
  VARIANT 39: note; note (original language) = 能够与修饰物进行偶联，且在肿瘤微环境中能够与修饰物解偶联，释放多肽
PKKKIQLHAEHALXDALMILNIVKTNSPPAEEKLEDAXNFELILEEIARLFESGDQKDEAEKAKRMKEWMKRIKTTASEDEQEEMANAIITILQSWIFS